European Patent Application EP 4 293 047 A1, published December 20, 2023. Title: ANTI-PD-L1 ANTIBODY AND USE THEREOF. Applicant: SHANGHAI JEMINCARE PHARMACEUTICAL CO., LTD.; JIANGXI JEMINCARE GROUP CO., LTD. The sequence listing filed with the application follows.

SEQUENCE LISTING (63 sequences)

SEQ ID NO: 1 - protein, 7 aa, Artificial Sequence
  HCDR1
GFTFSNF

SEQ ID NO: 2 - protein, 6 aa, Artificial Sequence
  HCDR2
THSGGI

SEQ ID NO: 3 - protein, 9 aa, Artificial Sequence
  HCDR3
DPTEAPFDY

SEQ ID NO: 4 - protein, 11 aa, Artificial Sequence
  LCDR1
QASQNINNYIA

SEQ ID NO: 5 - protein, 7 aa, Artificial Sequence
  LCDR2
YTSTLVS

SEQ ID NO: 6 - protein, 9 aa, Artificial Sequence
  LCDR3
LQYDNVPNT

SEQ ID NO: 7 - protein, 25 aa, Artificial Sequence
  50G2-3 H-FR1
EVQLVESGGGLVQPGRSLKLSCVAS

SEQ ID NO: 8 - protein, 25 aa, Artificial Sequence [sequence omitted]

SEQ ID NO: 9 - protein, 19 aa, Artificial Sequence
  50G2-3 H-FR2
WMTWIRQAPGKGLEWVASI

SEQ ID NO: 10 - protein, 19 aa, Artificial Sequence
  1910G2HzH2, 1910G2HzH4 and 1910G2HzH7 H-FR2
WMTWVRQAPGKGLEWVASI

SEQ ID NO: 11 - protein, 19 aa, Artificial Sequence
  1910G2HzH3 and 1910G2HzH9 H-FR2
WMSWVRQAPGKGLEWVASI

SEQ ID NO: 12 - protein, 41 aa, Artificial Sequence
  50G2-3 H-FR3
TYYPDSVKGRFTISRDDAKSTLYLQMNSLRSEDTATYYCSR

SEQ ID NO: 13 - protein, 41 aa, Artificial Sequence
  1910G2HzH2 H-FR3
TYYVDSVKGRFTISRDDAKSSLYLQMNSLRAEDTAVYYCSR

SEQ ID NO: 14 - protein, 41 aa, Artificial Sequence
  1910G2HzH3 H-FR3
TYYVDSVKGRFTISRDNAKSSLYLQMNSLRAEDTAVYYCSR

SEQ ID NO: 15 - protein, 41 aa, Artificial Sequence
  1910G2HzH4 H-FR3
TYYPDSVKGRFTISRDDSKNTLYLQMNSLRAEDTAVYYCSR

SEQ ID NO: 16 - protein, 41 aa, Artificial Sequence
  1910G2HzH7 H-FR3
TYYADSVKGRFTISRDDSKSTLYLQMNSLRAEDTAVYYCSR

SEQ ID NO: 17 - protein, 41 aa, Artificial Sequence
  1910G2HzH9 H-FR3
TYYADSVKGRFTISRDDSKNTLYLQMNSLRAEDTAVYYCSR

SEQ ID NO: 18 - protein, 11 aa, Artificial Sequence
  50G2-3 and 1910G2HzH3 H-FR4
WGQGVMVTVSS

SEQ ID NO: 19 - protein, 11 aa, Artificial Sequence
  1910G2HzH2, 1910G2HzH4, 1910G2HzH7 and 1910G2HzH9 H-FR4
WGQGTLVTVSS

SEQ ID NO: 20 - protein, 118 aa, Artificial Sequence
  50G2-3 VH
EVQLVESGGGLVQPGRSLKLSCVASGFTFSNFWMTWIRQAPGKGLEWVASITHSGGITYYPDSVKGRFTISRDDAKSTLYLQMNSLRSEDTATYYCSRDPTEAPFDYWGQGVMVTVSS

SEQ ID NO: 21 - protein, 118 aa, Artificial Sequence
  1910G2HzH2 VH
EVQLVESGGGLVQPGGSLRLSCAASGFTFSNFWMTWVRQAPGKGLEWVASITHSGGITYYVDSVKGRFTISRDDAKSSLYLQMNSLRAEDTAVYYCSRDPTEAPFDYWGQGTLVTVSS

SEQ ID NO: 22 - protein, 118 aa, Artificial Sequence
  1910G2HzH3 VH
EVQLVESGGGLVQPGGSLRLSCAASGFTFSNFWMSWVRQAPGKGLEWVASITHSGGITYYVDSVKGRFTISRDNAKSSLYLQMNSLRAEDTAVYYCSRDPTEAPFDYWGQGVMVTVSS

SEQ ID NO: 23 - protein, 118 aa, Artificial Sequence
  1910G2HzH4 VH
EVQLVESGGGLVQPGGSLRLSCAASGFTFSNFWMTWVRQAPGKGLEWVASITHSGGITYYPDSVKGRFTISRDDSKNTLYLQMNSLRAEDTAVYYCSRDPTEAPFDYWGQGTLVTVSS

SEQ ID NO: 24 - protein, 118 aa, Artificial Sequence
  1910G2HzH7 VH
EVQLVESGGGLVQPGGSLRLSCAASGFTFSNFWMTWVRQAPGKGLEWVASITHSGGITYYADSVKGRFTISRDDSKSTLYLQMNSLRAEDTAVYYCSRDPTEAPFDYWGQGTLVTVSS

SEQ ID NO: 25 - protein, 118 aa, Artificial Sequence
  1910G2HzH9 VH
EVQLVESGGGLVQPGGSLRLSCAASGFTFSNFWMSWVRQAPGKGLEWVASITHSGGITYYADSVKGRFTISRDDSKNTLYLQMNSLRAEDTAVYYCSRDPTEAPFDYWGQGTLVTVSS

SEQ ID NO: 26 - protein, 23 aa, Artificial Sequence
  50G2-3 L-FR1
DIQMTQSPPSLSASLGDQVTITC

SEQ ID NO: 27 - protein, 23 aa, Artificial Sequence
  1910G2HzL2, 1910G2HzL3 and 1910G2HzL9 L-FR1
DIQMTQSPSSLSASVGDRVTITC

SEQ ID NO: 28 - protein, 15 aa, Artificial Sequence
  50G2-3 L-FR2
WYQQKPGKAPRQLIR

SEQ ID NO: 29 - protein, 15 aa, Artificial Sequence
  1910G2HzL2, 1910G2HzL3 and 1910G2HzL9 L-FR2
WYQQKPGKAPKQLIR

SEQ ID NO: 30 - protein, 32 aa, Artificial Sequence
  50G2-3 L-FR3
GTPSRFSGSGSGKDYSFSISNVESEDIASYYC

SEQ ID NO: 31 - protein, 32 aa, Artificial Sequence
  1910G2HzL2 L-FR3
GVPSRFSGSGSGKDYTFTISSLQPEDIATYYC

SEQ ID NO: 32 - protein, 32 aa, Artificial Sequence
  1910G2HzL3 L-FR3
GTPSRFSGSGSGKDYTFTISNLQPEDIATYYC

SEQ ID NO: 33 - protein, 32 aa, Artificial Sequence
  1910G2HzL9 L-FR3
GVPSRFSGSGSGKDFTFTISSLQPEDIATYYC

SEQ ID NO: 34 - protein, 10 aa, Artificial Sequence
  50G2-3 L-FR4
FGAGTKLELK

SEQ ID NO: 35 - protein, 10 aa, Artificial Sequence
  1910G2HzL2, 1910G2HzL3 and 1910G2HzL9 L-FR4
FGQGTKLEIK

SEQ ID NO: 36 - protein, 107 aa, Artificial Sequence
  50G2-3 VL
DIQMTQSPPSLSASLGDQVTITCQASQNINNYIAWYQQKPGKAPRQLIRYTSTLVSGTPSRFSGSGSGKDYSFSISNVESEDIASYYCLQYDNVPNTFGAGTKLELK

SEQ ID NO: 37 - protein, 107 aa, Artificial Sequence
  1910G2HzL2 VL
DIQMTQSPSSLSASVGDRVTITCQASQNINNYIAWYQQKPGKAPKQLIRYTSTLVSGVPSRFSGSGSGKDYTFTISSLQPEDIATYYCLQYDNVPNTFGQGTKLEIK

SEQ ID NO: 38 - protein, 107 aa, Artificial Sequence
  1910G2HzL3 VL
DIQMTQSPSSLSASVGDRVTITCQASQNINNYIAWYQQKPGKAPKQLIRYTSTLVSGTPSRFSGSGSGKDYTFTISNLQPEDIATYYCLQYDNVPNTFGQGTKLEIK

SEQ ID NO: 39 - protein, 107 aa, Artificial Sequence
  1910G2HzL9 VL
DIQMTQSPSSLSASVGDRVTITCQASQNINNYIAWYQQKPGKAPKQLIRYTSTLVSGVPSRFSGSGSGKDFTFTISSLQPEDIATYYCLQYDNVPNTFGQGTKLEIK

SEQ ID NO: 40 - protein, 107 aa, Artificial Sequence [sequence omitted]

SEQ ID NO: 41 - protein, 330 aa, Artificial Sequence
  Heavy Chain Constant Region
ASTKGPSVFPLAPSSKSTSGGTAALGCLVKDYFPEPVTVSWNSGALTSGVHTFPAVLQSSGLYSLSSVVTVPSSSLGTQTYICNVNHKPSNTKVDKKVEPKSCDKTHTCPPCPAPELLGGPSVFLFPPKPKDTLMISRTPEVTCVVVDVSHEDPEVKFNWYVDGVEVHNAKTKPREEQYASTYRVVSVLTVLHQDWLNGKEYKCKVSNKALPAPIEKTISKAKGQPREPQVYTLPPSREEMTKNQVSLTCLVKGFYPSDIAVEWESNGQPENNYKTTPPVLDSDGSFFLYSKLTVDKSRWQQGNVFSCSVMHEALHNHYTQKSLSLSPGK

SEQ ID NO: 42 - protein, 448 aa, Artificial Sequence
  1910G2HzH2 Heavy Chain
EVQLVESGGGLVQPGGSLRLSCAASGFTFSNFWMTWVRQAPGKGLEWVASITHSGGITYYVDSVKGRFTISRDDAKSSLYLQMNSLRAEDTAVYYCSRDPTEAPFDYWGQGTLVTVSSASTKGPSVFPLAPSSKSTSGGTAALGCLVKDYFPEPVTVSWNSGALTSGVHTFPAVLQSSGLYSLSSVVTVPSSSLGTQTYICNVNHKPSNTKVDKKVEPKSCDKTHTCPPCPAPELLGGPSVFLFPPKPKDTLMISRTPEVTCVVVDVSHEDPEVKFNWYVDGVEVHNAKTKPREEQYASTYRVVSVLTVLHQDWLNGKEYKCKVSNKALPAPIEKTISKAKGQPREPQVYTLPPSREEMTKNQVSLTCLVKGFYPSDIAVEWESNGQPENNYKTTPPVLDSDGSFFLYSKLTVDKSRWQQGNVFSCSVMHEALHNHYTQKSLSLSPGK

SEQ ID NO: 43 - protein, 448 aa, Artificial Sequence
  1910G2HzH3 Heavy Chain
EVQLVESGGGLVQPGGSLRLSCAASGFTFSNFWMSWVRQAPGKGLEWVASITHSGGITYYVDSVKGRFTISRDNAKSSLYLQMNSLRAEDTAVYYCSRDPTEAPFDYWGQGVMVTVSSASTKGPSVFPLAPSSKSTSGGTAALGCLVKDYFPEPVTVSWNSGALTSGVHTFPAVLQSSGLYSLSSVVTVPSSSLGTQTYICNVNHKPSNTKVDKKVEPKSCDKTHTCPPCPAPELLGGPSVFLFPPKPKDTLMISRTPEVTCVVVDVSHEDPEVKFNWYVDGVEVHNAKTKPREEQYASTYRVVSVLTVLHQDWLNGKEYKCKVSNKALPAPIEKTISKAKGQPREPQVYTLPPSREEMTKNQVSLTCLVKGFYPSDIAVEWESNGQPENNYKTTPPVLDSDGSFFLYSKLTVDKSRWQQGNVFSCSVMHEALHNHYTQKSLSLSPGK

SEQ ID NO: 44 - protein, 448 aa, Artificial Sequence
  1910G2HzH4 Heavy Chain
EVQLVESGGGLVQPGGSLRLSCAASGFTFSNFWMTWVRQAPGKGLEWVASITHSGGITYYPDSVKGRFTISRDDSKNTLYLQMNSLRAEDTAVYYCSRDPTEAPFDYWGQGTLVTVSSASTKGPSVFPLAPSSKSTSGGTAALGCLVKDYFPEPVTVSWNSGALTSGVHTFPAVLQSSGLYSLSSVVTVPSSSLGTQTYICNVNHKPSNTKVDKKVEPKSCDKTHTCPPCPAPELLGGPSVFLFPPKPKDTLMISRTPEVTCVVVDVSHEDPEVKFNWYVDGVEVHNAKTKPREEQYASTYRVVSVLTVLHQDWLNGKEYKCKVSNKALPAPIEKTISKAKGQPREPQVYTLPPSREEMTKNQVSLTCLVKGFYPSDIAVEWESNGQPENNYKTTPPVLDSDGSFFLYSKLTVDKSRWQQGNVFSCSVMHEALHNHYTQKSLSLSPGK

SEQ ID NO: 45 - protein, 448 aa, Artificial Sequence
  1910G2HzH7 Heavy Chain
EVQLVESGGGLVQPGGSLRLSCAASGFTFSNFWMTWVRQAPGKGLEWVASITHSGGITYYADSVKGRFTISRDDSKSTLYLQMNSLRAEDTAVYYCSRDPTEAPFDYWGQGTLVTVSSASTKGPSVFPLAPSSKSTSGGTAALGCLVKDYFPEPVTVSWNSGALTSGVHTFPAVLQSSGLYSLSSVVTVPSSSLGTQTYICNVNHKPSNTKVDKKVEPKSCDKTHTCPPCPAPELLGGPSVFLFPPKPKDTLMISRTPEVTCVVVDVSHEDPEVKFNWYVDGVEVHNAKTKPREEQYASTYRVVSVLTVLHQDWLNGKEYKCKVSNKALPAPIEKTISKAKGQPREPQVYTLPPSREEMTKNQVSLTCLVKGFYPSDIAVEWESNGQPENNYKTTPPVLDSDGSFFLYSKLTVDKSRWQQGNVFSCSVMHEALHNHYTQKSLSLSPGK

SEQ ID NO: 46 - protein, 448 aa, Artificial Sequence
  1910G2HzH9 Heavy Chain
EVQLVESGGGLVQPGGSLRLSCAASGFTFSNFWMSWVRQAPGKGLEWVASITHSGGITYYADSVKGRFTISRDDSKNTLYLQMNSLRAEDTAVYYCSRDPTEAPFDYWGQGTLVTVSSASTKGPSVFPLAPSSKSTSGGTAALGCLVKDYFPEPVTVSWNSGALTSGVHTFPAVLQSSGLYSLSSVVTVPSSSLGTQTYICNVNHKPSNTKVDKKVEPKSCDKTHTCPPCPAPELLGGPSVFLFPPKPKDTLMISRTPEVTCVVVDVSHEDPEVKFNWYVDGVEVHNAKTKPREEQYASTYRVVSVLTVLHQDWLNGKEYKCKVSNKALPAPIEKTISKAKGQPREPQVYTLPPSREEMTKNQVSLTCLVKGFYPSDIAVEWESNGQPENNYKTTPPVLDSDGSFFLYSKLTVDKSRWQQGNVFSCSVMHEALHNHYTQKSLSLSPGK

SEQ ID NO: 47 - protein, 214 aa, Artificial Sequence
  1910G2HzL2 Light Chain
DIQMTQSPSSLSASVGDRVTITCQASQNINNYIAWYQQKPGKAPKQLIRYTSTLVSGVPSRFSGSGSGKDYTFTISSLQPEDIATYYCLQYDNVPNTFGQGTKLEIKRTVAAPSVFIFPPSDEQLKSGTASVVCLLNNFYPREAKVQWKVDNALQSGNSQESVTEQDSKDSTYSLSSTLTLSKADYEKHKVYACEVTHQGLSSPVTKSFNRGEC

SEQ ID NO: 48 - protein, 214 aa, Artificial Sequence
  1910G2HzL3 Light Chain
DIQMTQSPSSLSASVGDRVTITCQASQNINNYIAWYQQKPGKAPKQLIRYTSTLVSGTPSRFSGSGSGKDYTFTISNLQPEDIATYYCLQYDNVPNTFGQGTKLEIKRTVAAPSVFIFPPSDEQLKSGTASVVCLLNNFYPREAKVQWKVDNALQSGNSQESVTEQDSKDSTYSLSSTLTLSKADYEKHKVYACEVTHQGLSSPVTKSFNRGEC

SEQ ID NO: 49 - protein, 214 aa, Artificial Sequence
  1910G2HzL9 Light Chain
DIQMTQSPSSLSASVGDRVTITCQASQNINNYIAWYQQKPGKAPKQLIRYTSTLVSGVPSRFSGSGSGKDFTFTISSLQPEDIATYYCLQYDNVPNTFGQGTKLEIKRTVAAPSVFIFPPSDEQLKSGTASVVCLLNNFYPREAKVQWKVDNALQSGNSQESVTEQDSKDSTYSLSSTLTLSKADYEKHKVYACEVTHQGLSSPVTKSFNRGEC

SEQ ID NO: 50 - protein, 25 aa, Artificial Sequence
  50G2-3 H-FR1; 1910G2HzH2, 1910G2HzH3, 1910G2HzH4, 1910G2HzH7 and 1910G2HzH9 H-FR1
  misc_feature (16)..(16): Xaa = Gly or Arg
  misc_feature (19)..(19): Xaa = Lys or Arg
  misc_feature (23)..(23): Xaa = Ala or Val
EVQLVESGGGLVQPGXSLXLSCXAS

SEQ ID NO: 51 - protein, 19 aa, Artificial Sequence
  50G2-3 H-FR2; 1910G2HzH2, 1910G2HzH4 and 1910G2HzH7 H-FR2; 1910G2HzH3 and 1910G2HzH9 H-FR2
  misc_feature (3)..(3): Xaa = Ser or Thr
  misc_feature (5)..(5): Xaa = Ile or Val
WMXWXRQAPGKGLEWVASI

SEQ ID NO: 52 - protein, 41 aa, Artificial Sequence
  50G2-3 H-FR3; 1910G2HzH2 H-FR3; 1910G2HzH3 H-FR3; 1910G2HzH4 H-FR3; 1910G2HzH7 H-FR3; 1910G2HzH9 H-FR3
  misc_feature (4)..(4): Xaa = Ala, Pro or Val
  misc_feature (17)..(17): Xaa = Asp or Asn
  misc_feature (18)..(18): Xaa = Ala or Ser
  misc_feature (20)..(20): Xaa = Asn or Ser
  misc_feature (21)..(21): Xaa = Ser or Thr
  misc_feature (31)..(31): Xaa = Ala or Ser
  misc_feature (36)..(36): Xaa = Thr or Val
TYYXDSVKGRFTISRDXXKXXLYLQMNSLRXEDTAXYYCSR

SEQ ID NO: 53 - protein, 11 aa, Artificial Sequence
  50G2-3 and 1910G2HzH3 H-FR4; 1910G2HzH2, 1910G2HzH4, 1910G2HzH7 and 1910G2HzH9 H-FR4
  misc_feature (5)..(5): Xaa = Thr or Val
  misc_feature (6)..(6): Xaa = Leu or Met
WGQGXXVTVSS

SEQ ID NO: 54 - protein, 118 aa, Artificial Sequence
  50G2-3 VH; 1910G2HzH2 VH; 1910G2HzH3 VH; 1910G2HzH4 VH; 1910G2HzH7 VH; 1910G2HzH9 VH
  misc_feature (16)..(16): Xaa = Gly or Arg
  misc_feature (19)..(19): Xaa = Lys or Arg
  misc_feature (23)..(23): Xaa = Ala or Val
  misc_feature (35)..(35): Xaa = Ser or Thr
  misc_feature (37)..(37): Xaa = Ile or Val
  misc_feature (61)..(61): Xaa = Ala, Pro or Val
  misc_feature (74)..(74): Xaa = Asp or Asn
  misc_feature (75)..(75): Xaa = Ala or Ser
  misc_feature (77)..(77): Xaa = Asn or Ser
  misc_feature (78)..(78): Xaa = Ser or Thr
  misc_feature (88)..(88): Xaa = Ala or Ser
  misc_feature (93)..(93): Xaa = Thr or Val
  misc_feature (112)..(112): Xaa = Thr or Val
  misc_feature (113)..(113): Xaa = Leu or Met
EVQLVESGGGLVQPGXSLXLSCXASGFTFSNFWMXWXRQAPGKGLEWVASITHSGGITYYXDSVKGRFTISRDXXKXXLYLQMNSLRXEDTAXYYCSRDPTEAPFDYWGQGXXVTVSS

SEQ ID NO: 55 - protein, 23 aa, Artificial Sequence
  50G2-3 L-FR1; 1910G2HzL2, 1910G2HzL3 and 1910G2HzL9 L-FR1
  misc_feature (9)..(9): Xaa = Pro or Ser
  misc_feature (15)..(15): Xaa = Leu or Val
  misc_feature (18)..(18): Xaa = Gln or Arg
DIQMTQSPXSLSASXGDXVTITC

SEQ ID NO: 56 - protein, 15 aa, Artificial Sequence
  50G2-3 L-FR2; 1910G2HzL2, 1910G2HzL3 and 1910G2HzL9 L-FR2
  misc_feature (11)..(11): Xaa = Lys or Arg
WYQQKPGKAPXQLIR

SEQ ID NO: 57 - protein, 32 aa, Artificial Sequence
  50G2-3 L-FR3; 1910G2HzL2 L-FR3; 1910G2HzL3 L-FR3; 1910G2HzL9 L-FR3
  misc_feature (2)..(2): Xaa = Thr or Val
  misc_feature (15)..(15): Xaa = Phe or Tyr
  misc_feature (16)..(16): Xaa = Ser or Thr
  misc_feature (18)..(18): Xaa = Ser or Thr
  misc_feature (21)..(21): Xaa = Asn or Ser
  misc_feature (22)..(22): Xaa = Leu or Val
  misc_feature (23)..(23): Xaa = Glu or Gln
  misc_feature (24)..(24): Xaa = Pro or Ser
  misc_feature (29)..(29): Xaa = Ser or Thr
GXPSRFSGSGSGKDXXFXISXXXXEDIAXYYC

SEQ ID NO: 58 - protein, 10 aa, Artificial Sequence
  50G2-3 L-FR4; 1910G2HzL2, 1910G2HzL3 and 1910G2HzL9 L-FR4
  misc_feature (3)..(3): Xaa = Ala or Gln
  misc_feature (9)..(9): Xaa = Ile or Leu
FGXGTKLEXK

SEQ ID NO: 59 - protein, 107 aa, Artificial Sequence
  50G2-3 VL; 1910G2HzL2 VL; 1910G2HzL3 VL; 1910G2HzL9 VL
  misc_feature (9)..(9): Xaa = Pro or Ser
  misc_feature (15)..(15): Xaa = Leu or Val
  misc_feature (18)..(18): Xaa = Gln or Arg
  misc_feature (45)..(45): Xaa = Lys or Arg
  misc_feature (58)..(58): Xaa = Thr or Val
  misc_feature (71)..(71): Xaa = Phe or Tyr
  misc_feature (72)..(72): Xaa = Ser or Thr
  misc_feature (74)..(74): Xaa = Ser or Thr
  misc_feature (77)..(77): Xaa = Asn or Ser
  misc_feature (78)..(78): Xaa = Leu or Val
  misc_feature (79)..(79): Xaa = Glu or Gln
  misc_feature (80)..(80): Xaa = Pro or Ser
  misc_feature (85)..(85): Xaa = Ser or Thr
  misc_feature (100)..(100): Xaa = Ala or Gln
  misc_feature (106)..(106): Xaa = Ile or Leu
DIQMTQSPXSLSASXGDXVTITCQASQNINNYIAWYQQKPGKAPXQLIRYTSTLVSGXPSRFSGSGSGKDXXFXISXXXXEDIAXYYCLQYDNVPNTFGXGTKLEXK

SEQ ID NO: 60 - protein, 95 aa, Homo sapiens
DIQMTQSPSSLSASVGDRVTITCQASQDISNYLNWYQQKPGKAPKLLIYDASNLETGVPSRFSGSGSGTDFTFTISSLQPEDIATYYCQQYDNLP

SEQ ID NO: 61 - protein, 12 aa, Homo sapiens
YTFGQGTKLEIK

SEQ ID NO: 62 - protein, 98 aa, Homo sapiens
EVQLVESGGGLVQPGGSLRLSCAASGFTFSSYWMSWVRQAPGKGLEWVANIKQDGSEKYYVDSVKGRFTISRDNAKNSLYLQMNSLRAEDTAVYYCAR

SEQ ID NO: 63 - protein, 15 aa, Homo sapiens
YFDYWGQGTLVTVSS